European Patent Application EP 4 578 961 A2, published July 2, 2025. Title: SALIVARY BIOMARKERS OF BRAIN INJURY. Applicant: MARKER DIAGNOSTICS UK LIMITED. Application EP. The sequence listing filed with the application follows.

SEQUENCE LISTING (356 sequences)

SEQ ID NO: 1 - RNA, 22 nt, Homo sapiens
  source 1..22: mol_type = unassigned RNA
tagcttatcagactgatgttga

SEQ ID NO: 2 - RNA, 23 nt, Homo sapiens
  source 1..23: mol_type = unassigned RNA
aatgacacgatcactcccgttga

SEQ ID NO: 3-13 - skipped (11 entries)

SEQ ID NO: 14 - RNA, 21 nt, Homo sapiens
  source 1..21: mol_type = unassigned RNA
cattattacttttggtacgcg

SEQ ID NO: 15 - skipped

SEQ ID NO: 16 - RNA, 22 nt, Homo sapiens
  source 1..22: mol_type = unassigned RNA
ggatatcatcatatactgtaag

SEQ ID NO: 17-22 - skipped (6 entries)

SEQ ID NO: 23 - RNA, 21 nt, Homo sapiens
  source 1..21: mol_type = unassigned RNA
tccggttctcagggctccacc

SEQ ID NO: 24-25 - skipped (2 entries)

SEQ ID NO: 26 - RNA, 23 nt, Homo sapiens
  source 1..23: mol_type = unassigned RNA
tgtagtgtttcctactttatgga

SEQ ID NO: 27 - RNA, 22 nt, Homo sapiens
  source 1..22: mol_type = unassigned RNA
tcagtgcactacagaactttgt

SEQ ID NO: 28 - skipped

SEQ ID NO: 29 - RNA, 22 nt, Homo sapiens
  source 1..22: mol_type = unassigned RNA
tgaggtagtagtttgtgctgtt

SEQ ID NO: 30-38 - skipped (9 entries)

SEQ ID NO: 39 - RNA, 23 nt, Homo sapiens
  source 1..23: mol_type = unassigned RNA
agcagcattgtacagggctatca

SEQ ID NO: 40 - DNA, 23 bp, Homo sapiens
  source 1..23: mol_type = unassigned DNA
tatggcttttcattcctatgtga

SEQ ID NO: 41-47 - skipped (7 entries)

SEQ ID NO: 48 - DNA, 21 bp, Homo sapiens
  source 1..21: mol_type = unassigned DNA
tgagatgaagcactgtagctc

SEQ ID NO: 49-69 - skipped (21 entries)

SEQ ID NO: 70 - DNA, 21 bp, Homo sapiens
  source 1..21: mol_type = unassigned DNA
ggagaatagaacatgctgatt

SEQ ID NO: 71 - DNA, 18 bp, Homo sapiens
  source 1..18: mol_type = unassigned DNA
ataacgtcatctagtgtg

SEQ ID NO: 72 - DNA, 18 bp, Homo sapiens
  source 1..18: mol_type = unassigned DNA
cacgagagaacgcacacc

SEQ ID NO: 73 - DNA, 21 bp, Homo sapiens
  source 1..21: mol_type = unassigned DNA
gaccttgggttgggtcgtggt

SEQ ID NO: 74 - DNA, 18 bp, Homo sapiens
  source 1..18: mol_type = unassigned DNA
ataaggaactgctctctc

SEQ ID NO: 75 - DNA, 16 bp, Homo sapiens
  source 1..16: mol_type = unassigned DNA
gtggtcaggtagagaa

SEQ ID NO: 76 - DNA, 27 bp, Homo sapiens
  source 1..27: mol_type = unassigned DNA
gggtaaaactgcagtgggcgttggtag

SEQ ID NO: 77 - DNA, 16 bp, Homo sapiens
  source 1..16: mol_type = unassigned DNA
cagggctgtgctaact

SEQ ID NO: 78 - DNA, 17 bp, Homo sapiens
  source 1..17: mol_type = unassigned DNA
gcggaccttgctcaagg

SEQ ID NO: 79 - DNA, 18 bp, Homo sapiens
  source 1..18: mol_type = unassigned DNA
gtgaaaagacataggggg

SEQ ID NO: 80 - DNA, 17 bp, Homo sapiens
  source 1..17: mol_type = unassigned DNA
aggaccattgcgttgcc

SEQ ID NO: 81 - DNA, 18 bp, Homo sapiens
  source 1..18: mol_type = unassigned DNA
agagactgactttgagta

SEQ ID NO: 82 - DNA, 17 bp, Homo sapiens
  source 1..17: mol_type = unassigned DNA
aaatggcgatactcagg

SEQ ID NO: 83 - DNA, 17 bp, Homo sapiens
  source 1..17: mol_type = unassigned DNA
tggattgtgggggaacc

SEQ ID NO: 84 - DNA, 16 bp, Homo sapiens
  source 1..16: mol_type = unassigned DNA
caactgtaagtccatt

SEQ ID NO: 85 - DNA, 16 bp, Homo sapiens
  source 1..16: mol_type = unassigned DNA
ggtcctcggatcggcc

SEQ ID NO: 86 - DNA, 16 bp, Homo sapiens
  source 1..16: mol_type = unassigned DNA
tagcttgatccagttg

SEQ ID NO: 87 - DNA, 16 bp, Homo sapiens
  source 1..16: mol_type = unassigned DNA
tgtggattgatgctct

SEQ ID NO: 88 - DNA, 16 bp, Homo sapiens
  source 1..16: mol_type = unassigned DNA
caagagatgaggaatg

SEQ ID NO: 89 - DNA, 16 bp, Homo sapiens
  source 1..16: mol_type = unassigned DNA
tggacttcagaacagc

SEQ ID NO: 90 - DNA, 18 bp, Homo sapiens
  source 1..18: mol_type = unassigned DNA
aaggcgaaggatatgttg

SEQ ID NO: 91 - DNA, 22 bp, Homo sapiens
  source 1..22: mol_type = unassigned DNA
tgtctactactggagacactgg

SEQ ID NO: 92 - DNA, 21 bp, Homo sapiens
  source 1..21: mol_type = unassigned DNA
cataaagtagaaagcactact

SEQ ID NO: 93 - DNA, 21 bp, Homo sapiens
  source 1..21: mol_type = unassigned DNA
tcctgtccctgtctcctacag

SEQ ID NO: 94 - DNA, 22 bp, Homo sapiens
  source 1..22: mol_type = unassigned DNA
cttggcacctagcaagcactca

SEQ ID NO: 95 - DNA, 22 bp, Homo sapiens
  source 1..22: mol_type = unassigned DNA
caatcactaactccactgccat

SEQ ID NO: 96 - DNA, 22 bp, Homo sapiens
  source 1..22: mol_type = unassigned DNA
tggcagtgtattgttagctggt

SEQ ID NO: 97 - DNA, 50 bp, Homo sapiens
  source 1..50: mol_type = unassigned DNA
aagattagcatgaggatgacacgcaaattcgtgaagcgttccatttcttt

SEQ ID NO: 98 - DNA, 50 bp, Homo sapiens
  source 1..50: mol_type = unassigned DNA
ggcccctgcacagggatgacacgcaaattcgtgaagcgttccatattttt

SEQ ID NO: 99 - DNA, 50 bp, Homo sapiens
  source 1..50: mol_type = unassigned DNA
ggcccctgcgcaaggatgacatgcaaattcgtgaagcgttccatattttt

SEQ ID NO: 100 - DNA, 50 bp, Homo sapiens
  source 1..50: mol_type = unassigned DNA
ggcccctgtgcaaggatgacacgcaaattcgtgaagcgttccatattttt

SEQ ID NO: 101 - DNA, 50 bp, Homo sapiens
  source 1..50: mol_type = unassigned DNA
ggcccttgtgcaaggatgacacgcaaattcgtgaagcgttccatattttt

SEQ ID NO: 102 - DNA, 50 bp, Homo sapiens
  source 1..50: mol_type = unassigned DNA
ggcccctgtgcaaggatgacatgcaaattcgtgaagcgttccatattttt

SEQ ID NO: 103 - RNA, 50 nt, Homo sapiens
  source 1..50: mol_type = unassigned RNA
gtgtcaccaacgttggtatacaaccccccacaactaaatttgactggctt

SEQ ID NO: 104 - DNA, 50 bp, Homo sapiens
  source 1..50: mol_type = unassigned DNA
ggcccctgtgcaagaatgactcgcaaattcgtgaagcgttccatattttt

SEQ ID NO: 105 - DNA, 50 bp, Homo sapiens
  source 1..50: mol_type = unassigned DNA
gatggcatgacccctgatcaaggacggcatgcaaatttgtgaagtatttc

SEQ ID NO: 106 - RNA, 22 nt, Homo sapiens
  source 1..22: mol_type = unassigned RNA
tgaggtagtaggttgtatagtt

SEQ ID NO: 107 - RNA, 22 nt, Homo sapiens
  source 1..22: mol_type = unassigned RNA
tgaggtagtaggttgtgtggtt

SEQ ID NO: 108 - RNA, 22 nt, Homo sapiens
  source 1..22: mol_type = unassigned RNA
tgaggtagtagattgtatagtt

SEQ ID NO: 109 - RNA, 23 nt, Homo sapiens
  source 1..23: mol_type = unassigned RNA
agcagcattgtacagggctatga

SEQ ID NO: 110 - RNA, 19 nt, Homo sapiens
  source 1..19: mol_type = unassigned RNA
aatggatttttggagcagg

SEQ ID NO: 111 - RNA, 22 nt, Homo sapiens
  source 1..22: mol_type = unassigned RNA
tcgtaccgtgagtaataatgcg

SEQ ID NO: 112 - RNA, 21 nt, Homo sapiens
  source 1..21: mol_type = unassigned RNA
cataaagtagaaagcactact

SEQ ID NO: 113 - RNA, 20 nt, Homo sapiens
  source 1..20: mol_type = unassigned RNA
tacagtatagatgatgtact

SEQ ID NO: 114 - RNA, 22 nt, Homo sapiens
  source 1..22: mol_type = unassigned RNA
ccagtattaactgtgctgctga

SEQ ID NO: 115 - RNA, 22 nt, Homo sapiens
  source 1..22: mol_type = unassigned RNA
tggaatgtaaggaagtgtgtgg

SEQ ID NO: 116 - RNA, 22 nt, Homo sapiens
  source 1..22: mol_type = unassigned RNA
tagcaccatttgaaatcggtta

SEQ ID NO: 117 - RNA, 23 nt, Homo sapiens
  source 1..23: mol_type = unassigned RNA
tccctgtcctccaggagctcacg

SEQ ID NO: 118 - RNA, 22 nt, Homo sapiens
  source 1..22: mol_type = unassigned RNA
caatcactaactccactgccat

SEQ ID NO: 119 - RNA, 22 nt, Homo sapiens
  source 1..22: mol_type = unassigned RNA
tggcagtgtattgttagctggt

SEQ ID NO: 120 - RNA, 21 nt, Homo sapiens
  source 1..21: mol_type = unassigned RNA
cagcagcacactgtggtttgt

SEQ ID NO: 121 - RNA, 21 nt, Homo sapiens
  source 1..21: mol_type = unassigned RNA
tcctgtccctgtctcctacag

SEQ ID NO: 122 - RNA, 22 nt, Homo sapiens
  source 1..22: mol_type = unassigned RNA
tattgcacttgtcccggcctgt

SEQ ID NO: 123 - RNA, 22 nt, Homo sapiens
  source 1..22: mol_type = unassigned RNA
tgtctactactggagacactgg

SEQ ID NO: 124 - DNA, 17 bp, Homo sapiens
  source 1..17: mol_type = unassigned DNA
agggctgggcacggggg

SEQ ID NO: 125 - DNA, 18 bp, Homo sapiens
  source 1..18: mol_type = unassigned DNA
ataaaatgggcgttgagg

SEQ ID NO: 126 - DNA, 23 bp, Homo sapiens
  source 1..23: mol_type = unassigned DNA
ttcaaatcccacttctgacacca

SEQ ID NO: 127 - DNA, 23 bp, Homo sapiens
  source 1..23: mol_type = unassigned DNA
ctgaaaaggggacggattgggaa

SEQ ID NO: 128 - DNA, 19 bp, Homo sapiens
  source 1..19: mol_type = unassigned DNA
ccagttgtcgtgggttttt

SEQ ID NO: 129 - DNA, 22 bp, Homo sapiens
  source 1..22: mol_type = unassigned DNA
gcgggggattagctcagctggg

SEQ ID NO: 130 - DNA, 17 bp, Homo sapiens
  source 1..17: mol_type = unassigned DNA
tgattttttttggcgaa

SEQ ID NO: 131 - DNA, 18 bp, Homo sapiens
  source 1..18: mol_type = unassigned DNA
aaggatagggaggtattt

SEQ ID NO: 132 - DNA, 17 bp, Homo sapiens
  source 1..17: mol_type = unassigned DNA
accatcctctgctacca

SEQ ID NO: 133 - DNA, 17 bp, Homo sapiens
  source 1..17: mol_type = unassigned DNA
acagggctgtgcaaaaa

SEQ ID NO: 134 - DNA, 50 bp, Homo sapiens
  source 1..50: mol_type = unassigned DNA
tatcgtagccaatgaggtttatccgaggcgtgattattgctaattgaaaa

SEQ ID NO: 135 - DNA, 50 bp, Homo sapiens
  source 1..50: mol_type = unassigned DNA
tgctggcggcttcccatccgctggttctatcctcaaacgccgggacaccg

SEQ ID NO: 136 - DNA, 50 bp, Homo sapiens
  source 1..50: mol_type = unassigned DNA
cttctctccgtattggggagtgagagggagagaacgcggtctgagtggtt

SEQ ID NO: 137 - DNA, 50 bp, Homo sapiens
  source 1..50: mol_type = unassigned DNA
gcgcatgcttagcatgcatgaggtcccgggttcgatccccagcatctcca

SEQ ID NO: 138 - DNA, 50 bp, Homo sapiens
  source 1..50: mol_type = unassigned DNA
gcactggcctcctaagccagggattgtgggttcgagtcccacctggggta

SEQ ID NO: 139 - DNA, 50 bp, Homo sapiens
  source 1..50: mol_type = unassigned DNA
gcgtcagtctcataatctgaaggtcctgagttcgagcctcagagagggca

SEQ ID NO: 140 - DNA, 50 bp, Homo sapiens
  source 1..50: mol_type = unassigned DNA
gcataaaacttaaaattttataatcagaggttcaactcctcttcttaaca

SEQ ID NO: 141 - DNA, 50 bp, Homo sapiens
  source 1..50: mol_type = unassigned DNA
gcgtctgattccggatcagaagattgagggttcgagtcccttcgtggtcg

SEQ ID NO: 142 - DNA, 50 bp, Homo sapiens
  source 1..50: mol_type = unassigned DNA
gcgcctgtctagtaaacaggagatcctgggttcgaatcccagcggtgcct

SEQ ID NO: 143 - DNA, 50 bp, Homo sapiens
  source 1..50: mol_type = unassigned DNA
ctttttgactgtagagcaagaggtccctggttcaaatccaggttctccct

SEQ ID NO: 144 - DNA, 50 bp, Homo sapiens
  source 1..50: mol_type = unassigned DNA
tcacttcacgcatcgatctggtattgcagtacctccaggaacagtgcacc

SEQ ID NO: 145 - DNA, 50 bp, Homo sapiens
  source 1..50: mol_type = unassigned DNA
gtatcgtagccaatgaggtttatccaaggtgcgattattgctaattgaaa

SEQ ID NO: 146 - DNA, 50 bp, Homo sapiens
  source 1..50: mol_type = unassigned DNA
atggcccctgcgcaaggatgacacgcaaatttgtgaaggattccatattt

SEQ ID NO: 147 - DNA, 50 bp, Homo sapiens
  source 1..50: mol_type = unassigned DNA
ggcccctgcgcaaggatgacatgcaaatttgtgaagtgttccatattttt

SEQ ID NO: 148 - DNA, 30 bp, Homo sapiens
  source 1..30: mol_type = unassigned DNA
cattgatcatcgacacttcgaacgcacttg

SEQ ID NO: 149 - DNA, 50 bp, Homo sapiens
  source 1..50: mol_type = unassigned DNA
gtctttgttgaactctttccctccttctcattactgtacttgaccagtct

SEQ ID NO: 150 - DNA, 50 bp, Homo sapiens
  source 1..50: mol_type = unassigned DNA
gcttcttttactctttcccttcattctcactactgtacctgattcgtctt

SEQ ID NO: 151 - RNA, 23 nt, Homo sapiens
  source 1..23: mol_type = unassigned RNA
tatggcttttcattcctatgtga

SEQ ID NO: 152 - RNA, 21 nt, Homo sapiens
  source 1..21: mol_type = unassigned RNA
tgagatgaagcactgtagctc

SEQ ID NO: 153 - protein, 4 aa, unidentified
  REGION 1..4: note = source = /note="Description of Unknown: 'DEVD' caspase-3 inhibitor sequence"
DEVD

SEQ ID NO: 154 - DNA, 16 bp, Homo sapiens
  source 1..16: mol_type = unassigned DNA
ttcaggttaccgcagg

SEQ ID NO: 155 - DNA, 17 bp, Homo sapiens
  source 1..17: mol_type = unassigned DNA
gactgctcgagctgctt

SEQ ID NO: 156 - DNA, 16 bp, Homo sapiens
  source 1..16: mol_type = unassigned DNA
tgggcagcaagaatgg

SEQ ID NO: 157 - DNA, 16 bp, Homo sapiens
  source 1..16: mol_type = unassigned DNA
ggaggatttcaattgg

SEQ ID NO: 158 - DNA, 16 bp, Homo sapiens
  source 1..16: mol_type = unassigned DNA
tctgtcatggctgagc

SEQ ID NO: 159 - DNA, 17 bp, Homo sapiens
  source 1..17: mol_type = unassigned DNA
tacctcaattctctagg

SEQ ID NO: 160 - DNA, 20 bp, Homo sapiens
  source 1..20: mol_type = unassigned DNA
tgtcggcgggggccccggac

SEQ ID NO: 161 - DNA, 17 bp, Homo sapiens
  source 1..17: mol_type = unassigned DNA
cattctctgaaactaca

SEQ ID NO: 162 - DNA, 16 bp, Homo sapiens
  source 1..16: mol_type = unassigned DNA
gacttgtgattagcgg

SEQ ID NO: 163 - DNA, 18 bp, Homo sapiens
  source 1..18: mol_type = unassigned DNA
gagcatgttgactggaga

SEQ ID NO: 164 - DNA, 17 bp, Homo sapiens
  source 1..17: mol_type = unassigned DNA
tgagaaaacatttgagg

SEQ ID NO: 165 - DNA, 18 bp, Homo sapiens
  source 1..18: mol_type = unassigned DNA
ccaggctggtcgtgatga

SEQ ID NO: 166 - DNA, 21 bp, Homo sapiens
  source 1..21: mol_type = unassigned DNA
tcggaagaagaagctgaccca

SEQ ID NO: 167 - DNA, 19 bp, Homo sapiens
  source 1..19: mol_type = unassigned DNA
taactcttggaaatcttgg

SEQ ID NO: 168 - DNA, 20 bp, Homo sapiens
  source 1..20: mol_type = unassigned DNA
aaaaaagagggacagaaatg

SEQ ID NO: 169 - DNA, 18 bp, Homo sapiens
  source 1..18: mol_type = unassigned DNA
gaaaagcaatcgtcacag

SEQ ID NO: 170 - DNA, 21 bp, Homo sapiens
  source 1..21: mol_type = unassigned DNA
aatattcagcagtcagactgg

SEQ ID NO: 171 - DNA, 17 bp, Homo sapiens
  source 1..17: mol_type = unassigned DNA
cagggtgatgacttctg

SEQ ID NO: 172 - DNA, 23 bp, Homo sapiens
  source 1..23: mol_type = unassigned DNA
gtgatgtcggctcatcgcaacct

SEQ ID NO: 173 - DNA, 27 bp, Homo sapiens
  source 1..27: mol_type = unassigned DNA
tgagggatgtttggatgctcgctttga

SEQ ID NO: 174 - DNA, 17 bp, Homo sapiens
  source 1..17: mol_type = unassigned DNA
taattgtcctcttgggg

SEQ ID NO: 175 - DNA, 17 bp, Homo sapiens
  source 1..17: mol_type = unassigned DNA
aagcaggcgttacaatg

SEQ ID NO: 176 - DNA, 20 bp, Homo sapiens
  source 1..20: mol_type = unassigned DNA
tgaactcgggagaaggaagt

SEQ ID NO: 177 - DNA, 19 bp, Homo sapiens
  source 1..19: mol_type = unassigned DNA
cctgtctgactgggtctcc

SEQ ID NO: 178 - DNA, 19 bp, Homo sapiens
  source 1..19: mol_type = unassigned DNA
aagaagtagactggattgg

SEQ ID NO: 179 - DNA, 18 bp, Homo sapiens
  source 1..18: mol_type = unassigned DNA
taagtgggagtgctcatg

SEQ ID NO: 180 - DNA, 16 bp, Homo sapiens
  source 1..16: mol_type = unassigned DNA
gttaagtatgcacagg

SEQ ID NO: 181 - DNA, 18 bp, Homo sapiens
  source 1..18: mol_type = unassigned DNA
tggcatcctgtctcttgc

SEQ ID NO: 182 - DNA, 21 bp, Homo sapiens
  source 1..21: mol_type = unassigned DNA
cacgctgtcttttgtttctct

SEQ ID NO: 183 - DNA, 19 bp, Homo sapiens
  source 1..19: mol_type = unassigned DNA
tggaagaggggaaaggaga

SEQ ID NO: 184 - DNA, 17 bp, Homo sapiens
  source 1..17: mol_type = unassigned DNA
ctaagagtatgagtagc

SEQ ID NO: 185 - DNA, 17 bp, Homo sapiens
  source 1..17: mol_type = unassigned DNA
tcaggacattggactct

SEQ ID NO: 186 - DNA, 22 bp, Homo sapiens
  source 1..22: mol_type = unassigned DNA
gagaagactgaatgctcttctc

SEQ ID NO: 187 - DNA, 19 bp, Homo sapiens
  source 1..19: mol_type = unassigned DNA
gctggaatagctcagttgc

SEQ ID NO: 188 - DNA, 20 bp, Homo sapiens
  source 1..20: mol_type = unassigned DNA
cagcatcatgatcattatgg

SEQ ID NO: 189 - DNA, 27 bp, Homo sapiens
  source 1..27: mol_type = unassigned DNA
cattgtgcttcgtgggagagtagggca

SEQ ID NO: 190 - DNA, 18 bp, Homo sapiens
  source 1..18: mol_type = unassigned DNA
gccgacaggtccgggtaa

SEQ ID NO: 191 - DNA, 18 bp, Homo sapiens
  source 1..18: mol_type = unassigned DNA
tagattcaggaactgcca

SEQ ID NO: 192 - DNA, 21 bp, Homo sapiens
  source 1..21: mol_type = unassigned DNA
tttagtagaattgtgttgggt

SEQ ID NO: 193 - DNA, 18 bp, Homo sapiens
  source 1..18: mol_type = unassigned DNA
aaaagcaaggcgaagagg

SEQ ID NO: 194 - DNA, 20 bp, Homo sapiens
  source 1..20: mol_type = unassigned DNA
cagactgctcgagctgctgc

SEQ ID NO: 195 - DNA, 17 bp, Homo sapiens
  source 1..17: mol_type = unassigned DNA
tttgcagactggaaact

SEQ ID NO: 196 - DNA, 18 bp, Homo sapiens
  source 1..18: mol_type = unassigned DNA
tgtctgtagcaatgtgct

SEQ ID NO: 197 - DNA, 17 bp, Homo sapiens
  source 1..17: mol_type = unassigned DNA
tggggataaagttaggt

SEQ ID NO: 198 - DNA, 16 bp, Homo sapiens
  source 1..16: mol_type = unassigned DNA
tggctgttgcacttct

SEQ ID NO: 199 - DNA, 17 bp, Homo sapiens
  source 1..17: mol_type = unassigned DNA
ttgaagactggctctca

SEQ ID NO: 200 - DNA, 17 bp, Homo sapiens
  source 1..17: mol_type = unassigned DNA
caacggtcttgaaaaca

SEQ ID NO: 201 - DNA, 17 bp, Homo sapiens
  source 1..17: mol_type = unassigned DNA
tggaagaaaacgaggag

SEQ ID NO: 202 - DNA, 17 bp, Homo sapiens
  source 1..17: mol_type = unassigned DNA
attttggtctgttggtt

SEQ ID NO: 203 - DNA, 21 bp, Homo sapiens
  source 1..21: mol_type = unassigned DNA
atgtaaccgggcttttgtgct

SEQ ID NO: 204 - DNA, 19 bp, Homo sapiens
  source 1..19: mol_type = unassigned DNA
caggcagaagggagcttgt

SEQ ID NO: 205 - DNA, 17 bp, Homo sapiens
  source 1..17: mol_type = unassigned DNA
cacgttcttctcatggt

SEQ ID NO: 206 - DNA, 17 bp, Homo sapiens
  source 1..17: mol_type = unassigned DNA
aaagttgtgttagctga

SEQ ID NO: 207 - DNA, 18 bp, Homo sapiens
  source 1..18: mol_type = unassigned DNA
tatgattgtaaactctga

SEQ ID NO: 208 - DNA, 26 bp, Homo sapiens
  source 1..26: mol_type = unassigned DNA
cacatgggggtagagcactgactggg

SEQ ID NO: 209 - DNA, 18 bp, Homo sapiens
  source 1..18: mol_type = unassigned DNA
ctgcaggagtgtttgaga

SEQ ID NO: 210 - DNA, 17 bp, Homo sapiens
  source 1..17: mol_type = unassigned DNA
caaatgatcaaagcagg

SEQ ID NO: 211 - DNA, 17 bp, Homo sapiens
  source 1..17: mol_type = unassigned DNA
atcggaaaatgtgggaa

SEQ ID NO: 212 - DNA, 17 bp, Homo sapiens
  source 1..17: mol_type = unassigned DNA
aaatgcattggatatgg

SEQ ID NO: 213 - DNA, 17 bp, Homo sapiens
  source 1..17: mol_type = unassigned DNA
gttgtaaagctctgttg

SEQ ID NO: 214 - DNA, 21 bp, Homo sapiens
  source 1..21: mol_type = unassigned DNA
gttctgagttctttggttgga

SEQ ID NO: 215 - DNA, 20 bp, Homo sapiens
  source 1..20: mol_type = unassigned DNA
ttcactactttatctctttt

SEQ ID NO: 216 - DNA, 27 bp, Homo sapiens
  source 1..27: mol_type = unassigned DNA
agactgtgatgactgggagagcgggct

SEQ ID NO: 217 - DNA, 19 bp, Homo sapiens
  source 1..19: mol_type = unassigned DNA
gaggctcgagagcaatggc

SEQ ID NO: 218 - DNA, 20 bp, Homo sapiens
  source 1..20: mol_type = unassigned DNA
aagttggagtatgttttagg

SEQ ID NO: 219 - DNA, 16 bp, Homo sapiens
  source 1..16: mol_type = unassigned DNA
ccatgactgcagatgg

SEQ ID NO: 220 - DNA, 18 bp, Homo sapiens
  source 1..18: mol_type = unassigned DNA
ctggagatctgtttgggc

SEQ ID NO: 221 - DNA, 17 bp, Homo sapiens
  source 1..17: mol_type = unassigned DNA
gtggggcttagtgctga

SEQ ID NO: 222 - DNA, 16 bp, Homo sapiens
  source 1..16: mol_type = unassigned DNA
gggatcaacctgacaa

SEQ ID NO: 223 - DNA, 18 bp, Homo sapiens
  source 1..18: mol_type = unassigned DNA
ccaacagcttctgagttg

SEQ ID NO: 224 - DNA, 18 bp, Homo sapiens
  source 1..18: mol_type = unassigned DNA
gtcctgtgtcttgtacgg

SEQ ID NO: 225 - DNA, 17 bp, Homo sapiens
  source 1..17: mol_type = unassigned DNA
agaggacagggaagctt

SEQ ID NO: 226 - DNA, 18 bp, Homo sapiens
  source 1..18: mol_type = unassigned DNA
agaagtcagaacctctat

SEQ ID NO: 227 - DNA, 19 bp, Homo sapiens
  source 1..19: mol_type = unassigned DNA
gacagattttagcttgtcc

SEQ ID NO: 228 - DNA, 19 bp, Homo sapiens
  source 1..19: mol_type = unassigned DNA
taacaggcgttgaaattgt

SEQ ID NO: 229 - DNA, 19 bp, Homo sapiens
  source 1..19: mol_type = unassigned DNA
gatgggggtagagcactgc

SEQ ID NO: 230 - DNA, 18 bp, Homo sapiens
  source 1..18: mol_type = unassigned DNA
tggggattgtgggttctc

SEQ ID NO: 231 - DNA, 16 bp, Homo sapiens
  source 1..16: mol_type = unassigned DNA
agaggacagggaagct

SEQ ID NO: 232 - DNA, 27 bp, Homo sapiens
  source 1..27: mol_type = unassigned DNA
agagggttcctgtagacctagggagga

SEQ ID NO: 233 - DNA, 23 bp, Homo sapiens
  source 1..23: mol_type = unassigned DNA
agccagagttctgattgtgagtg

SEQ ID NO: 234 - DNA, 18 bp, Homo sapiens
  source 1..18: mol_type = unassigned DNA
tgagttctttggtcagaa

SEQ ID NO: 235 - DNA, 19 bp, Homo sapiens
  source 1..19: mol_type = unassigned DNA
agtagctggtcgatttggc

SEQ ID NO: 236 - DNA, 19 bp, Homo sapiens
  source 1..19: mol_type = unassigned DNA
cttcagactgtgaaactga

SEQ ID NO: 237 - DNA, 17 bp, Homo sapiens
  source 1..17: mol_type = unassigned DNA
tagagatagagcttatg

SEQ ID NO: 238 - DNA, 18 bp, Homo sapiens
  source 1..18: mol_type = unassigned DNA
tggagacattaactatga

SEQ ID NO: 239 - DNA, 16 bp, Homo sapiens
  source 1..16: mol_type = unassigned DNA
tgggaagggctgccgg

SEQ ID NO: 240 - DNA, 17 bp, Homo sapiens
  source 1..17: mol_type = unassigned DNA
ttggtagactctcactt

SEQ ID NO: 241 - DNA, 18 bp, Homo sapiens
  source 1..18: mol_type = unassigned DNA
tggataactctttttgta

SEQ ID NO: 242 - DNA, 17 bp, Homo sapiens
  source 1..17: mol_type = unassigned DNA
tatgggaagaatctggg

SEQ ID NO: 243 - DNA, 19 bp, Homo sapiens
  source 1..19: mol_type = unassigned DNA
tatgtcatggtggctttgg

SEQ ID NO: 244 - DNA, 20 bp, Homo sapiens
  source 1..20: mol_type = unassigned DNA
gaatcccacttctgacacca

SEQ ID NO: 245 - DNA, 19 bp, Homo sapiens
  source 1..19: mol_type = unassigned DNA
atggtctagagctacaggt

SEQ ID NO: 246 - DNA, 18 bp, Homo sapiens
  source 1..18: mol_type = unassigned DNA
cagcttcttccgcttctt

SEQ ID NO: 247 - DNA, 16 bp, Homo sapiens
  source 1..16: mol_type = unassigned DNA
gtactgcatctctgca

SEQ ID NO: 248 - DNA, 17 bp, Homo sapiens
  source 1..17: mol_type = unassigned DNA
actggatccaagaaaag

SEQ ID NO: 249 - DNA, 17 bp, Homo sapiens
  source 1..17: mol_type = unassigned DNA
aggacgttggtcagagc

SEQ ID NO: 250 - DNA, 17 bp, Homo sapiens
  source 1..17: mol_type = unassigned DNA
tctctcaatcctcttgg

SEQ ID NO: 251 - DNA, 17 bp, Homo sapiens
  source 1..17: mol_type = unassigned DNA
agaagcagagaacgagg

SEQ ID NO: 252 - DNA, 18 bp, Homo sapiens
  source 1..18: mol_type = unassigned DNA
aggagatatagctcttgt

SEQ ID NO: 253 - DNA, 17 bp, Homo sapiens
  source 1..17: mol_type = unassigned DNA
aaaatggattcgaacca

SEQ ID NO: 254 - DNA, 18 bp, Homo sapiens
  source 1..18: mol_type = unassigned DNA
tgaccttttgccttctgc

SEQ ID NO: 255 - DNA, 20 bp, Homo sapiens
  source 1..20: mol_type = unassigned DNA
taaaaagttctctgtttttc

SEQ ID NO: 256 - DNA, 21 bp, Homo sapiens
  source 1..21: mol_type = unassigned DNA
ttggtgcatctgtagtccaac

SEQ ID NO: 257 - DNA, 19 bp, Homo sapiens
  source 1..19: mol_type = unassigned DNA
tgaaattctaaatattgca

SEQ ID NO: 258 - DNA, 16 bp, Homo sapiens
  source 1..16: mol_type = unassigned DNA
tgggatttagctcagc

SEQ ID NO: 259 - DNA, 17 bp, Homo sapiens
  source 1..17: mol_type = unassigned DNA
aagtgggaaggcccaga

SEQ ID NO: 260 - DNA, 17 bp, Homo sapiens
  source 1..17: mol_type = unassigned DNA
tgctttgatcgtagccc

SEQ ID NO: 261 - DNA, 19 bp, Homo sapiens
  source 1..19: mol_type = unassigned DNA
gaggttaggatatctggct

SEQ ID NO: 262 - DNA, 18 bp, Homo sapiens
  source 1..18: mol_type = unassigned DNA
ttttgaacgttctttctt

SEQ ID NO: 263 - DNA, 20 bp, Homo sapiens
  source 1..20: mol_type = unassigned DNA
aaggggaggaatttcacgtg

SEQ ID NO: 264 - DNA, 16 bp, Homo sapiens
  source 1..16: mol_type = unassigned DNA
aaggaaaaagcggata

SEQ ID NO: 265 - DNA, 16 bp, Homo sapiens
  source 1..16: mol_type = unassigned DNA
tggtggagtgaagacg

SEQ ID NO: 266 - DNA, 17 bp, Homo sapiens
  source 1..17: mol_type = unassigned DNA
tggagtgtggattgggg

SEQ ID NO: 267 - DNA, 17 bp, Homo sapiens
  source 1..17: mol_type = unassigned DNA
ctgcgtggctctgacac

SEQ ID NO: 268 - DNA, 17 bp, Homo sapiens
  source 1..17: mol_type = unassigned DNA
aggtaaagctcatgagg

SEQ ID NO: 269 - DNA, 21 bp, Homo sapiens
  source 1..21: mol_type = unassigned DNA
ccaaggggttgtagggccact

SEQ ID NO: 270 - DNA, 16 bp, Homo sapiens
  source 1..16: mol_type = unassigned DNA
agactcctttatcgta

SEQ ID NO: 271 - DNA, 17 bp, Homo sapiens
  source 1..17: mol_type = unassigned DNA
atgagcattgatttagg

SEQ ID NO: 272 - DNA, 19 bp, Homo sapiens
  source 1..19: mol_type = unassigned DNA
ttgagatttgagggggcct

SEQ ID NO: 273 - DNA, 26 bp, Homo sapiens
  source 1..26: mol_type = unassigned DNA
ctgtgaagcctgttggtttgctgctg

SEQ ID NO: 274 - DNA, 18 bp, Homo sapiens
  source 1..18: mol_type = unassigned DNA
tgctgaacctctgtatgt

SEQ ID NO: 275 - DNA, 19 bp, Homo sapiens
  source 1..19: mol_type = unassigned DNA
cagggagtgaaagagaatt

SEQ ID NO: 276 - DNA, 17 bp, Homo sapiens
  source 1..17: mol_type = unassigned DNA
gaagttaaatccttggg

SEQ ID NO: 277 - DNA, 18 bp, Homo sapiens
  source 1..18: mol_type = unassigned DNA
attctttgacatgcagat

SEQ ID NO: 278 - DNA, 17 bp, Homo sapiens
  source 1..17: mol_type = unassigned DNA
ctggtgtagaattgagg

SEQ ID NO: 279 - DNA, 18 bp, Homo sapiens
  source 1..18: mol_type = unassigned DNA
caggtttcagactttagg

SEQ ID NO: 280 - DNA, 18 bp, Homo sapiens
  source 1..18: mol_type = unassigned DNA
tgtggatttttgtcatgt

SEQ ID NO: 281 - DNA, 20 bp, Homo sapiens
  source 1..20: mol_type = unassigned DNA
ccttgatctgactgggggcc

SEQ ID NO: 282 - DNA, 26 bp, Homo sapiens
  source 1..26: mol_type = unassigned DNA
ctgttggagaatttggaatattaggt

SEQ ID NO: 283 - DNA, 25 bp, Homo sapiens
  source 1..25: mol_type = unassigned DNA
gaagagggagtggtctgtaaatgcg

SEQ ID NO: 284 - DNA, 20 bp, Homo sapiens
  source 1..20: mol_type = unassigned DNA
aaagggaaacaagaattctt

SEQ ID NO: 285 - DNA, 19 bp, Homo sapiens
  source 1..19: mol_type = unassigned DNA
taaatgttggtttgtttgt

SEQ ID NO: 286 - DNA, 17 bp, Homo sapiens
  source 1..17: mol_type = unassigned DNA
gagcgaaacggcaggat

SEQ ID NO: 287 - DNA, 17 bp, Homo sapiens
  source 1..17: mol_type = unassigned DNA
acccggagaactgaact

SEQ ID NO: 288 - DNA, 17 bp, Homo sapiens
  source 1..17: mol_type = unassigned DNA
atttgaaagaatgcttg

SEQ ID NO: 289 - DNA, 18 bp, Homo sapiens
  source 1..18: mol_type = unassigned DNA
ctagctgaacctctgtat

SEQ ID NO: 290 - DNA, 21 bp, Homo sapiens
  source 1..21: mol_type = unassigned DNA
tgagctttggaagaaggacca

SEQ ID NO: 291 - DNA, 26 bp, Homo sapiens
  source 1..26: mol_type = unassigned DNA
tgtgaggatgttctgtaaggagtgtt

SEQ ID NO: 292 - DNA, 24 bp, Homo sapiens
  source 1..24: mol_type = unassigned DNA
tgaattacggaagtgttggttaat

SEQ ID NO: 293 - DNA, 19 bp, Homo sapiens
  source 1..19: mol_type = unassigned DNA
aagaggggcttttagaacc

SEQ ID NO: 294 - DNA, 18 bp, Homo sapiens
  source 1..18: mol_type = unassigned DNA
cgtggtgatgctctgaca

SEQ ID NO: 295 - DNA, 18 bp, Homo sapiens
  source 1..18: mol_type = unassigned DNA
ttgggaagggctgccgga

SEQ ID NO: 296 - DNA, 17 bp, Homo sapiens
  source 1..17: mol_type = unassigned DNA
atctcgatccagtagtc

SEQ ID NO: 297 - DNA, 19 bp, Homo sapiens
  source 1..19: mol_type = unassigned DNA
tttagaccgtttttatgtc

SEQ ID NO: 298 - DNA, 18 bp, Homo sapiens
  source 1..18: mol_type = unassigned DNA
tttgtagaagaggaagcg

SEQ ID NO: 299 - DNA, 18 bp, Homo sapiens
  source 1..18: mol_type = unassigned DNA
tagaatggggcttgttgc

SEQ ID NO: 300 - DNA, 20 bp, Homo sapiens
  source 1..20: mol_type = unassigned DNA
aaagaatgaagttggtctgg

SEQ ID NO: 301 - DNA, 17 bp, Homo sapiens
  source 1..17: mol_type = unassigned DNA
taatgaatgactgtttg

SEQ ID NO: 302 - DNA, 16 bp, Homo sapiens
  source 1..16: mol_type = unassigned DNA
aaagaacgttcaaagg

SEQ ID NO: 303 - DNA, 18 bp, Homo sapiens
  source 1..18: mol_type = unassigned DNA
aaagggctttgactattt

SEQ ID NO: 304 - DNA, 16 bp, Homo sapiens
  source 1..16: mol_type = unassigned DNA
tgcttcctcaatcggt

SEQ ID NO: 305 - DNA, 18 bp, Homo sapiens
  source 1..18: mol_type = unassigned DNA
acagtagcaatgttctgc

SEQ ID NO: 306 - DNA, 21 bp, Homo sapiens
  source 1..21: mol_type = unassigned DNA
gattatgattgtgattgtagc

SEQ ID NO: 307 - DNA, 17 bp, Homo sapiens
  source 1..17: mol_type = unassigned DNA
aaaaagttagacttagg

SEQ ID NO: 308 - DNA, 17 bp, Homo sapiens
  source 1..17: mol_type = unassigned DNA
gccaggatgttggctta

SEQ ID NO: 309 - DNA, 24 bp, Homo sapiens
  source 1..24: mol_type = unassigned DNA
ggaactcatgattgttgactttgg

SEQ ID NO: 310 - DNA, 16 bp, Homo sapiens
  source 1..16: mol_type = unassigned DNA
ttagaggccactcaat

SEQ ID NO: 311 - DNA, 23 bp, Homo sapiens
  source 1..23: mol_type = unassigned DNA
tatttaaatgagaactttgaagc

SEQ ID NO: 312 - DNA, 17 bp, Homo sapiens
  source 1..17: mol_type = unassigned DNA
cgttttggtgttggttg

SEQ ID NO: 313 - DNA, 18 bp, Homo sapiens
  source 1..18: mol_type = unassigned DNA
agaaccaagaagctctgg

SEQ ID NO: 314 - DNA, 19 bp, Homo sapiens
  source 1..19: mol_type = unassigned DNA
tagaagagggagcttcttt

SEQ ID NO: 315 - DNA, 16 bp, Homo sapiens
  source 1..16: mol_type = unassigned DNA
agagctagaatccagg

SEQ ID NO: 316 - DNA, 20 bp, Homo sapiens
  source 1..20: mol_type = unassigned DNA
tttattagagacgggacttt

SEQ ID NO: 317 - DNA, 19 bp, Homo sapiens
  source 1..19: mol_type = unassigned DNA
aaaggatgtagacaaggga

SEQ ID NO: 318 - DNA, 17 bp, Homo sapiens
  source 1..17: mol_type = unassigned DNA
caaatgaatatctggga

SEQ ID NO: 319 - DNA, 18 bp, Homo sapiens
  source 1..18: mol_type = unassigned DNA
tttaggtactctgaacaa

SEQ ID NO: 320 - DNA, 19 bp, Homo sapiens
  source 1..19: mol_type = unassigned DNA
cacagaaggaacgtttaga

SEQ ID NO: 321 - DNA, 18 bp, Homo sapiens
  source 1..18: mol_type = unassigned DNA
gaaagagagtgagactca

SEQ ID NO: 322 - DNA, 17 bp, Homo sapiens
  source 1..17: mol_type = unassigned DNA
tggtggttggttttggg

SEQ ID NO: 323 - DNA, 16 bp, Homo sapiens
  source 1..16: mol_type = unassigned DNA
attgtgaatgatctgg

SEQ ID NO: 324 - DNA, 20 bp, Homo sapiens
  source 1..20: mol_type = unassigned DNA
gcactctggactctgaatcc

SEQ ID NO: 325 - DNA, 16 bp, Homo sapiens
  source 1..16: mol_type = unassigned DNA
ttaggagtaggttact

SEQ ID NO: 326 - DNA, 20 bp, Homo sapiens
  source 1..20: mol_type = unassigned DNA
tgactgttttatatgagtaa

SEQ ID NO: 327 - DNA, 21 bp, Homo sapiens
  source 1..21: mol_type = unassigned DNA
atcccggacgagcccccatta

SEQ ID NO: 328 - DNA, 24 bp, Homo sapiens
  source 1..24: mol_type = unassigned DNA
ttgaaactgatatactgtcttagg

SEQ ID NO: 329 - DNA, 19 bp, Homo sapiens
  source 1..19: mol_type = unassigned DNA
gatgggctgattgagggat

SEQ ID NO: 330 - DNA, 18 bp, Homo sapiens
  source 1..18: mol_type = unassigned DNA
atgaggctgagattgtcc

SEQ ID NO: 331 - DNA, 23 bp, Homo sapiens
  source 1..23: mol_type = unassigned DNA
aatgagaactttgaaggccgaag

SEQ ID NO: 332 - DNA, 16 bp, Homo sapiens
  source 1..16: mol_type = unassigned DNA
acagactgtctttggg

SEQ ID NO: 333 - DNA, 22 bp, Homo sapiens
  source 1..22: mol_type = unassigned DNA
gaaattattgatccagtcacga

SEQ ID NO: 334 - DNA, 16 bp, Homo sapiens
  source 1..16: mol_type = unassigned DNA
gaagagttgatccatg

SEQ ID NO: 335 - DNA, 19 bp, Homo sapiens
  source 1..19: mol_type = unassigned DNA
gttttgggttgagtgagga

SEQ ID NO: 336 - DNA, 19 bp, Homo sapiens
  source 1..19: mol_type = unassigned DNA
gtctatttggattatcgtc

SEQ ID NO: 337 - DNA, 22 bp, Homo sapiens
  source 1..22: mol_type = unassigned DNA
gtttgaattgggaagctggggg

SEQ ID NO: 338 - DNA, 20 bp, Homo sapiens
  source 1..20: mol_type = unassigned DNA
cagttggtagagcacctgac

SEQ ID NO: 339 - DNA, 27 bp, Homo sapiens
  source 1..27: mol_type = unassigned DNA
cagtataattaggggttaattgtggga

SEQ ID NO: 340 - DNA, 16 bp, Homo sapiens
  source 1..16: mol_type = unassigned DNA
tggagtgtggattggg

SEQ ID NO: 341 - DNA, 17 bp, Homo sapiens
  source 1..17: mol_type = unassigned DNA
tgagtggtcaatggggg

SEQ ID NO: 342 - DNA, 18 bp, Homo sapiens
  source 1..18: mol_type = unassigned DNA
tgggctcaagctttctct

SEQ ID NO: 343 - DNA, 20 bp, Homo sapiens
  source 1..20: mol_type = unassigned DNA
tttagggttttaaggtgtta

SEQ ID NO: 344 - DNA, 19 bp, Homo sapiens
  source 1..19: mol_type = unassigned DNA
ggactgagagctctttctg

SEQ ID NO: 345 - DNA, 17 bp, Homo sapiens
  source 1..17: mol_type = unassigned DNA
gtgctgcatggctgtca

SEQ ID NO: 346 - DNA, 17 bp, Homo sapiens
  source 1..17: mol_type = unassigned DNA
gagatttacgacctagg

SEQ ID NO: 347 - DNA, 17 bp, Homo sapiens
  source 1..17: mol_type = unassigned DNA
tggctctgacactagta

SEQ ID NO: 348 - DNA, 19 bp, Homo sapiens
  source 1..19: mol_type = unassigned DNA
gaagtggaaggactatgaa

SEQ ID NO: 349 - DNA, 21 bp, Homo sapiens
  source 1..21: mol_type = unassigned DNA
agagacaggaactttgatttt

SEQ ID NO: 350 - DNA, 25 bp, Homo sapiens
  source 1..25: mol_type = unassigned DNA
aggctgagactggacagaaagacct

SEQ ID NO: 351 - DNA, 17 bp, Homo sapiens
  source 1..17: mol_type = unassigned DNA
gcctgcccggtgctggt

SEQ ID NO: 352 - DNA, 16 bp, Homo sapiens
  source 1..16: mol_type = unassigned DNA
gcgtgtgcgcgggagg

SEQ ID NO: 353 - DNA, 19 bp, Homo sapiens
  source 1..19: mol_type = unassigned DNA
caggtgaaatcgtggatgt

SEQ ID NO: 354 - DNA, 19 bp, Homo sapiens
  source 1..19: mol_type = unassigned DNA
tgatgcgttgggatgtagc

SEQ ID NO: 355 - DNA, 17 bp, Homo sapiens
  source 1..17: mol_type = unassigned DNA
ttaggaagctgctgatt

SEQ ID NO: 356 - DNA, 16 bp, Homo sapiens
  source 1..16: mol_type = unassigned DNA
ataggagacttctatc